European Patent Application EP 4 368 633 A1, published May 15, 2024. Title: DEIMMUNIZED FLAGELLIN AND VACCINE COMPOSITION COMPRISING THE SAME. Applicant: METACEN THERAPEUTICS. The sequence listing filed with the application follows.

SEQUENCE LISTING (1 sequence)

SEQ ID NO: 1 - protein, 19 aa, Artificial Sequence
  B-cell epitope in the variable region of FlaB
SYQAEEGKDKNWNVAAGDN